European Patent Specification EP 3 565 575 B1, published March 8, 2023. Title: ANG (1-7) DERVIATIVE OLIGOPEPTIDES FOR THE TREATMENT OF PAIN. Applicant: ARIZONA BOARD OF REGENTS ON BEHALF OF THE UNIVERSITY OF ARIZONA. Application PCT/US2018/012893. The sequence listing filed with the application follows.

SEQUENCE LISTING (27 sequences)

SEQ ID NO: 1 - protein, 8 aa, Artificial Sequence
  Description of Artificial Sequence: Synthetic peptide
  MOD_RES (1)..(1): Aspartic acid, glutamic acid, alanine or a glycosylated form thereof
  MOD_RES (2)..(2): Arginine, histidine, lysine or a glycosylated form thereof
  MOD_RES (3)..(3): Valine, alanine, isoleucine, leucine or a glycosylated form thereof
  MOD_RES (4)..(4): Tyrosine, phenylalanine, tryptophan or a glycosylated form thereof
  MOD_RES (5)..(5): Isoleucine, valine, alanine, leucine or a glycosylated form thereof
  MOD_RES (6)..(6): Histidine, arginine, lysine or a glycosylated form thereof
  MOD_RES (7)..(7): Proline, glycine, serine or a glycosylated form thereof
  MOD_RES (8)..(8): Can be absent or serine, threonine, hydroxyproline or a glycosylated form thereof
  See specification as filed for detailed description of substitutions and preferred embodiments
XXXXXXXX

SEQ ID NO: 2 - protein, 7 aa, Homo sapiens
DRVYIHP

SEQ ID NO: 3 - protein, 7 aa, Artificial Sequence
  Description of Artificial Sequence: Synthetic peptide
  MISC_FEATURE (7)..(7): Glycosylated
DRVYIHP

SEQ ID NO: 4 - protein, 7 aa, Artificial Sequence
  Description of Artificial Sequence: Synthetic peptide
  MISC_FEATURE (7)..(7): Carboxy terminal NH2
DRVYIHP

SEQ ID NO: 5 - protein, 7 aa, Artificial Sequence
  Description of Artificial Sequence: Synthetic peptide
  MISC_FEATURE (7)..(7): Glycosylated
  MISC_FEATURE (7)..(7): Carboxy terminal NH2
DRVYIHP

SEQ ID NO: 6 - protein, 8 aa, Artificial Sequence
  Description of Artificial Sequence: Synthetic peptide
DRVYIHPS

SEQ ID NO: 7 - protein, 8 aa, Artificial Sequence
  Description of Artificial Sequence: Synthetic peptide
  MISC_FEATURE (8)..(8): Glycosylated
DRVYIHPS

SEQ ID NO: 8 - protein, 8 aa, Artificial Sequence
  Description of Artificial Sequence: Synthetic peptide
  MISC_FEATURE (8)..(8): Carboxy terminal NH2
DRVYIHPS

SEQ ID NO: 9 - protein, 8 aa, Artificial Sequence
  Description of Artificial Sequence: Synthetic peptide
  MISC_FEATURE (8)..(8): Glycosylated
  MISC_FEATURE (8)..(8): Carboxy terminal NH2
  See specification as filed for detailed description of substitutions and preferred embodiments
DRVYIHPS

SEQ ID NO: 10 - protein, 7 aa, Artificial Sequence
  Description of Artificial Sequence: Synthetic peptide
DRVYIHS

SEQ ID NO: 11 - protein, 7 aa, Artificial Sequence
  Description of Artificial Sequence: Synthetic peptide
  MISC_FEATURE (7)..(7): Glycosylated
DRVYIHS

SEQ ID NO: 12 - protein, 7 aa, Artificial Sequence
  Description of Artificial Sequence: Synthetic peptide
  MISC_FEATURE (7)..(7): Carboxy terminal NH2
DRVYIHS

SEQ ID NO: 13 - protein, 7 aa, Artificial Sequence
  Description of Artificial Sequence: Synthetic peptide
  MISC_FEATURE (7)..(7): Glycosylated
  MISC_FEATURE (7)..(7): Carboxy terminal NH2
  See specification as filed for detailed description of substitutions and preferred embodiments
DRVYIHS

SEQ ID NO: 14 - protein, 7 aa, Artificial Sequence
  Description of Artificial Sequence: Synthetic peptide
ARVYIHP

SEQ ID NO: 15 - protein, 7 aa, Artificial Sequence
  Description of Artificial Sequence: Synthetic peptide
  MISC_FEATURE (7)..(7): Glycosylated
ARVYIHP

SEQ ID NO: 16 - protein, 7 aa, Artificial Sequence
  Description of Artificial Sequence: Synthetic peptide
  MISC_FEATURE (7)..(7): Carboxy terminal NH2
ARVYIHP

SEQ ID NO: 17 - protein, 7 aa, Artificial Sequence
  Description of Artificial Sequence: Synthetic peptide
  MISC_FEATURE (7)..(7): Glycosylated
  MISC_FEATURE (7)..(7): Carboxy terminal NH2
ARVYIHP

SEQ ID NO: 18 - protein, 8 aa, Artificial Sequence
  Description of Artificial Sequence: Synthetic peptide
ARVYIHPS

SEQ ID NO: 19 - protein, 8 aa, Artificial Sequence
  Description of Artificial Sequence: Synthetic peptide
  MISC_FEATURE (8)..(8): Glycosylated
ARVYIHPS

SEQ ID NO: 20 - protein, 8 aa, Artificial Sequence
  Description of Artificial Sequence: Synthetic peptide
  MISC_FEATURE (8)..(8): Carboxy terminal NH2
ARVYIHPS

SEQ ID NO: 21 - protein, 8 aa, Artificial Sequence
  Description of Artificial Sequence: Synthetic peptide
  MISC_FEATURE (8)..(8): Glycosylated
  MISC_FEATURE (8)..(8): Carboxy terminal NH2
ARVYIHPS

SEQ ID NO: 22 - protein, 7 aa, Artificial Sequence
  Description of Artificial Sequence: Synthetic peptide
ARVYIHS

SEQ ID NO: 23 - protein, 7 aa, Artificial Sequence
  Description of Artificial Sequence: Synthetic peptide
  MISC_FEATURE (7)..(7): Glycosylated
ARVYIHS

SEQ ID NO: 24 - protein, 7 aa, Artificial Sequence
  Description of Artificial Sequence: Synthetic peptide
  MISC_FEATURE (7)..(7): Carboxy terminal NH2
ARVYIHS

SEQ ID NO: 25 - protein, 7 aa, Artificial Sequence
  Description of Artificial Sequence: Synthetic peptide
  MISC_FEATURE (7)..(7): Glycosylated
  MISC_FEATURE (7)..(7): Carboxy terminal NH2
ARVYIHS

SEQ ID NO: 26 - protein, 7 aa, Artificial Sequence
  Description of Artificial Sequence: Synthetic peptide
  MOD_RES (1)..(1): Asp, Glu, Ala, Asn, Pro or Gly
  MISC_FEATURE (1)..(1): May be unmodified or may be glycosylated
  MOD_RES (2)..(2): Arg, Lys or Ala
  MISC_FEATURE (2)..(2): May be unmodified or may be glycosylated
  MOD_RES (3)..(3): Nle, Val, Leu, Ile, Ala, Gly, Lys, Pro or Tyr
  MISC_FEATURE (3)..(3): May be unmodified or may be glycosylated
  MOD_RES (4)..(4): Tyr, Ser, Thr or Ala
  MISC_FEATURE (4)..(4): May be unmodified or may be glycosylated
  MOD_RES (5)..(5): Ile, Val, Leu, Nle, Ala or Gly
  MOD_RES (6)..(6): His or Arg
  MISC_FEATURE (6)..(6): May be unmodified or may be glycosylated
  MOD_RES (7)..(7): Pro, Ser or Cys
  MISC_FEATURE (7)..(7): May be unmodified, may be glycosylated, may have a carboxy terminal NH2 or may be both glycosylated and have a carboxy terminal NH2
  See specification as filed for detailed description of substitutions and preferred embodiments
XXXXXXX

SEQ ID NO: 27 - protein, 8 aa, Artificial Sequence
  Description of Artificial Sequence: Synthetic peptide
  MOD_RES (1)..(1): Asp, Glu, Ala, Asn, Pro or Gly
  MISC_FEATURE (1)..(1): May be unmodified or may be glycosylated
  MOD_RES (2)..(2): Arg, Lys or Ala
  MISC_FEATURE (2)..(2): May be unmodified or may be glycosylated
  MOD_RES (3)..(3): Nle, Val, Leu, Ile, Ala, Gly, Lys, Pro or Tyr
  MISC_FEATURE (3)..(3): May be unmodified or may be glycosylated
  MOD_RES (4)..(4): Tyr, Ser, Thr or Ala
  MISC_FEATURE (4)..(4): May be unmodified or may be glycosylated
  MOD_RES (5)..(5): Ile, Val, Leu, Nle, Ala or Gly
  MOD_RES (6)..(6): His or Arg
  MISC_FEATURE (6)..(6): May be unmodified or may be glycosylated
  MOD_RES (7)..(7): Pro or Ala
  MOD_RES (8)..(8): Phe, Ser, Cys, Ile or Tyr
  MISC_FEATURE (8)..(8): May be unmodified, may be glycosylated, may have a carboxy terminal NH2 or may be both glycosylated and have a carboxy terminal NH2
  See specification as filed for detailed description of substitutions and preferred embodiments
XXXXXXXX